European Patent Specification EP 3 119 810 B1, published February 28, 2024. Title: METHODS FOR REDUCING CARDIOVASCULAR RISK. Applicant: BESSAC, Laurence HANOTIN, Corinne PORDY, Robert C. SASIELA, William J. SCHWARTZ, Gregory G. STEG, Philippe Gabriel. The sequence listing filed with the application follows.

SEQUENCE LISTING (198 sequences)

SEQ ID NO: 1 - protein, 118 aa, Artificial Sequence [sequence omitted]

SEQ ID NO: 2 - protein, 8 aa, Artificial Sequence
  Description of Artificial Sequence: Synthetic peptide
GFTFNNYA

SEQ ID NO: 3 - protein, 8 aa, Artificial Sequence
  Description of Artificial Sequence: Synthetic peptide
ISGSGGTT

SEQ ID NO: 4 - protein, 11 aa, Artificial Sequence
  Description of Artificial Sequence: Synthetic peptide
AKDSNWGNFDL

SEQ ID NO: 5 - protein, 447 aa, Artificial Sequence
  Description of Artificial Sequence: Synthetic REGN727 heavy chain polypeptide
EVQLVESGGGLVQPGGSLRLSCAASGFTFNNYAMNWVRQAPGKGLDWVSTISGSGGTTNYADSVKGRFIISRDSSKHTLYLQMNSLRAEDTAVYYCAKDSNWGNFDLWGRGTLVTVSSASTKGPSVFPLAPSSKSTSGGTAALGCLVKDYFPEPVTVSWNSGALTSGVHTFPAVLQSSGLYSLSSVVTVPSSSLGTQTYICNVNHKPSNTKVDKKVEPKSCDKTHTCPPCPAPELLGGPSVFLFPPKPKDTLMISRTPEVTCVVVDVSHEDPEVKFNWYVDGVEVHNAKTKPREEQYNSTYRVVSVLTVLHQDWLNGKEYKCKVSNKALPAPIEKTISKAKGQPREPQVYTLPPSRDELTKNQVSLTCLVKGFYPSDIAVEWESNGQPENNYKTTPPVLDSDGSFFLYSKLTVDKSRWQQGNVFSCSVMHEALHNHYTQKSLSLSPG

SEQ ID NO: 6 - protein, 113 aa, Artificial Sequence [sequence omitted]

SEQ ID NO: 7 - protein, 12 aa, Artificial Sequence
  Description of Artificial Sequence: Synthetic peptide
QSVLYRSNNRNF

SEQ ID NO: 8 - protein, 3 aa, Artificial Sequence
  Description of Artificial Sequence: Synthetic peptide
WAS

SEQ ID NO: 9 - protein, 220 aa, Artificial Sequence
  Description of Artificial Sequence: Synthetic REGN727 light chain polypeptide
DIVMTQSPDSLAVSLGERATINCKSSQSVLYRSNNRNFLGWYQQKPGQPPNLLIYWASTRESGVPDRFSGSGSGTDFTLTISSLQAEDVAVYYCQQYYTTPYTFGQGTKLEIKRTVAAPSVFIFPPSDEQLKSGTASVVCLLNNFYPREAKVQWKVDNALQSGNSQESVTEQDSKDSTYSLSSTLTLSKADYEKHKVYACEVTHQGLSSPVTKSFNRGEC

SEQ ID NO: 10 - protein, 9 aa, Artificial Sequence
  Description of Artificial Sequence: Synthetic peptide
QQYYTTPYT

SEQ ID NO: 11 - protein, 127 aa, Artificial Sequence
  Description of Artificial Sequence: Synthetic polypeptide
EMQLVESGGGLVQPGGSLRLSCAASGFTFSSHWMKWVRQAPGKGLEWVANINQDGSEKYYVDSVKGRFTISRDNAKNSLFLQMNSLRAEDTAVYYCARDIVLMVYDMDYYYYGMDVWGQGTTVTVSS

SEQ ID NO: 12 - protein, 8 aa, Artificial Sequence
  Description of Artificial Sequence: Synthetic peptide
GFTFSSHW

SEQ ID NO: 13 - protein, 8 aa, Artificial Sequence
  Description of Artificial Sequence: Synthetic peptide
INQDGSEK

SEQ ID NO: 14 - protein, 20 aa, Artificial Sequence
  Description of Artificial Sequence: Synthetic peptide
ARDIVLMVYDMDYYYYGMDV

SEQ ID NO: 15 - protein, 112 aa, Artificial Sequence
  Description of Artificial Sequence: Synthetic polypeptide
DIVMTQSPLSLPVTPGEPASISCRSSQSLLHSNGNNYLDWYLQKPGQSPQLLIYLGSNRASGVPDRFSGSGSGTDFTLKISRVEAEDVGVYYCMQTLQTPLTFGGGTKVEIK

SEQ ID NO: 16 - protein, 11 aa, Artificial Sequence
  Description of Artificial Sequence: Synthetic peptide
QSLLHSNGNNY

SEQ ID NO: 17 - protein, 3 aa, Artificial Sequence
  Description of Artificial Sequence: Synthetic peptide
LGS

SEQ ID NO: 18 - protein, 9 aa, Artificial Sequence
  Description of Artificial Sequence: Synthetic peptide
MQTLQTPLT

SEQ ID NO: 19 - protein, 8 aa, Artificial Sequence
  Description of Artificial Sequence: Synthetic peptide
GFTFSSHW

SEQ ID NO: 20 - protein, 8 aa, Artificial Sequence
  Description of Artificial Sequence: Synthetic peptide
INQDGSEK

SEQ ID NO: 21 - protein, 20 aa, Artificial Sequence
  Description of Artificial Sequence: Synthetic peptide
ARDIVLMVYDMDYYYYGMDV

SEQ ID NO: 22 - protein, 11 aa, Artificial Sequence
  Description of Artificial Sequence: Synthetic peptide
QSLHHSNGNNY

SEQ ID NO: 23 - protein, 3 aa, Artificial Sequence
  Description of Artificial Sequence: Synthetic peptide
LGS

SEQ ID NO: 24 - protein, 9 aa, Artificial Sequence
  Description of Artificial Sequence: Synthetic peptide
MQTLQTPLT

SEQ ID NO: 25 - protein, 8 aa, Artificial Sequence
  Description of Artificial Sequence: Synthetic peptide
GFTFSSHW

SEQ ID NO: 26 - protein, 8 aa, Artificial Sequence
  Description of Artificial Sequence: Synthetic peptide
INQDGSEK

SEQ ID NO: 27 - protein, 20 aa, Artificial Sequence
  Description of Artificial Sequence: Synthetic peptide
ARDIVLMVYHMDYYYYGMDV

SEQ ID NO: 28 - protein, 11 aa, Artificial Sequence
  Description of Artificial Sequence: Synthetic peptide
QSLLHSNGNNY

SEQ ID NO: 29 - protein, 3 aa, Artificial Sequence
  Description of Artificial Sequence: Synthetic peptide
LGS

SEQ ID NO: 30 - protein, 9 aa, Artificial Sequence
  Description of Artificial Sequence: Synthetic peptide
MQTLQTPLT

SEQ ID NO: 31 - protein, 8 aa, Artificial Sequence
  Description of Artificial Sequence: Synthetic peptide
GFTFSSHW

SEQ ID NO: 32 - protein, 8 aa, Artificial Sequence
  Description of Artificial Sequence: Synthetic peptide
INQDGSEK

SEQ ID NO: 33 - protein, 20 aa, Artificial Sequence
  Description of Artificial Sequence: Synthetic peptide
ARDIVLMVYHMDYYYYGMDV

SEQ ID NO: 34 - protein, 11 aa, Artificial Sequence
  Description of Artificial Sequence: Synthetic peptide
QSLHHSNGNNY

SEQ ID NO: 35 - protein, 3 aa, Artificial Sequence
  Description of Artificial Sequence: Synthetic peptide
LGS

SEQ ID NO: 36 - protein, 9 aa, Artificial Sequence
  Description of Artificial Sequence: Synthetic peptide
MQTLQTPLT

SEQ ID NO: 37 - protein, 131 aa, Artificial Sequence
  Description of Artificial Sequence: Synthetic VH; m2CX1D05 polypeptide
QVQLVQSGAEVKKPGSSVKVSCKASGGTFNSHAISWVRQAPGQGLEWMGGINPILGIANYAQKFQGRVTITADESTSTAYMELSSLRSEDTAVYYCARHYEIQIGRYGMNVYYLMYRFASWGQGTLVTVSS

SEQ ID NO: 38 - protein, 10 aa, Artificial Sequence
  Description of Artificial Sequence: Synthetic VH CDR1; m2CX1D05 peptide
GGTFNSHAIS

SEQ ID NO: 39 - protein, 20 aa, Artificial Sequence
  Description of Artificial Sequence: Synthetic VH CDR2; m2CX1D05 peptide
WMGGINPILGIANYAQKFQG

SEQ ID NO: 40 - protein, 22 aa, Artificial Sequence
  Description of Artificial Sequence: Synthetic VH CDR3; m2CX1D05 peptide
HYEIQIGRYGMNVYYLMYRFAS

SEQ ID NO: 41 - protein, 213 aa, Artificial Sequence
  Description of Artificial Sequence: Synthetic LC; m2CX1D05 polypeptide
DIQMTQSPSSLSASVGDRVTITCRASQGIRSALNWYQQKPGKAPKLLIYNGSTLQSGVPSRFSGSGSGTDFTLTISSLQPEDFAVYYCQQFDGDPTFGQGTKVEIKRTVAAPSVFIFPPSDEQLKSGTASVVCLLNNFYPREAKVQWKVDNALQSGNSQESVTEQDSKDSTYSLSSTLTLSKADYEKHKVYACEVTHQGLSSPVTKSFNRGEA

SEQ ID NO: 42 - protein, 11 aa, Artificial Sequence
  Description of Artificial Sequence: Synthetic VL CDR 1; m2CX1D05 peptide
RASQGIRSALN

SEQ ID NO: 43 - protein, 11 aa, Artificial Sequence
  Description of Artificial Sequence: Synthetic VL CDR2; m2CX1D05 peptide
LLIYNGSTLQS

SEQ ID NO: 44 - protein, 7 aa, Artificial Sequence
  Description of Artificial Sequence: Synthetic VL CDR3; m2CX1D05 peptide
QQFDGDP

SEQ ID NO: 45 - protein, 119 aa, Artificial Sequence
  Description of Artificial Sequence: Synthetic VH; 1B20 polypeptide
QVQLVQSGAEVKKPGESLKISCKGSGYSFTNYWISWVRQMPGKGLEWMGIIYPGDSYTNYSPSFQGQVTISADKSISTAYLQWSSLKASDTAMYYCARDYWYKPLFDIWGQGTLVTVSS

SEQ ID NO: 46 - protein, 10 aa, Artificial Sequence
  Description of Artificial Sequence: Synthetic VH CDR1; 1B20 peptide
GYSFTNYWIS

SEQ ID NO: 47 - protein, 20 aa, Artificial Sequence
  Description of Artificial Sequence: Synthetic VH CDR2; 1B20 peptide
WMGIIYPGDSYTNYSPSFQG

SEQ ID NO: 48 - protein, 10 aa, Artificial Sequence
  Description of Artificial Sequence: Synthetic VH CDR3; 1B20 peptide
DYWYKPLFDI

SEQ ID NO: 49 - protein, 220 aa, Artificial Sequence
  Description of Artificial Sequence: Synthetic LC; 1B20 polypeptide
DIVMTQSPDSLAVSLGERATINCRSSQSVLYSSNNKNYLAWYQQKPGQPPKLLIYWASTRESGVPDRFSGSGSGTDFTLTISSLQAEDVAVYYCQQYSSFPITFGQGTKVEIKRTVAAPSVFIFPPSDEQLKSGTASVVCLLNNFYPREAKVQWKVDNALQSGNSQESVTEQDSKDSTYSLSSTLTLSKADYEKHKVYACEVTHQGLSSPVTKSFNRGEA

SEQ ID NO: 50 - protein, 17 aa, Artificial Sequence
  Description of Artificial Sequence: Synthetic VL CDR1; 1B20 peptide
RSSQSVLYSSNNKNYLA

SEQ ID NO: 51 - protein, 11 aa, Artificial Sequence
  Description of Artificial Sequence: Synthetic VL CDR2; 1B20 peptide
LLIYWASTRES

SEQ ID NO: 52 - protein, 8 aa, Artificial Sequence
  Description of Artificial Sequence: Synthetic VL CDR3; 1B20 peptide
QQYSSFPI

SEQ ID NO: 53 - protein, 120 aa, Artificial Sequence
  Description of Artificial Sequence: Synthetic variable heavy antibody region polypeptide
EVQLLESGGGLVQPGGSLRLSCKASGYTFSSYGMYWVRQAPGKGLEWIGWIDPGSGGTKYNEKFKGKATISRDNSKNTLYLQMNSLRAEDTAVYYCARERYGYYFDYWGQGTLVTVSSAS

SEQ ID NO: 54 - protein, 16 aa, Artificial Sequence
  Description of Artificial Sequence: Synthetic AX132 heavy chain CDR1 antibody region peptide
KASGYTFSSYGMYWVR

SEQ ID NO: 55 - protein, 23 aa, Artificial Sequence
  Description of Artificial Sequence: Synthetic AX132 heavy chain CDR2 antibody region peptide
WIGWIDPGSGGTKYNEKFKGKAT

SEQ ID NO: 56 - protein, 15 aa, Artificial Sequence
  Description of Artificial Sequence: Synthetic AX132 heavy chain CDR3 antibody region peptide
CARERYGYYFDYWGQ

SEQ ID NO: 57 - protein, 108 aa, Artificial Sequence
  Description of Artificial Sequence: Synthetic variable light antibody region polypeptide
EIVLTQSPATLSLSPGERATITCRASQYVGSYLNWYQQKPGQAPRLLIYDASNRATGIPARFSGSGSGTDFTLTISSLEPEDFAVYYCQVWDSSPPVVFGGGTKVEIK

SEQ ID NO: 58 - protein, 17 aa, Artificial Sequence
  Description of Artificial Sequence: Synthetic AX213 and AX132 light chain CDR1 antibody region peptide
ITCRASQYVGSYLNWYQ

SEQ ID NO: 59 - protein, 13 aa, Artificial Sequence
  Description of Artificial Sequence: Synthetic AX213 and AX132 light chain CDR2 antibody region peptide
LIYDASNRATGIP

SEQ ID NO: 60 - protein, 16 aa, Artificial Sequence
  Description of Artificial Sequence: Synthetic AX132 & AX213 light chain CDR3 antibody region peptide
YYCQVWDSSPPVVFGG

SEQ ID NO: 61 - protein, 120 aa, Artificial Sequence
  Description of Artificial Sequence: Synthetic variable heavy antibody region polypeptide
EVQLLESGGGLVQPGGSLRLSCKASGYTFSRYGINWVRQAPGKGLEWIGRIDPGNGGTRYNEKFKGKATISRDNSKNTLYLQMNSLRAEDTAVYYCARANDGYSFDYWGQGTLVTVSSAS

SEQ ID NO: 62 - protein, 16 aa, Artificial Sequence
  Description of Artificial Sequence: Synthetic AX213 heavy chain CDR1 antibody region peptide
KASGYTFSRYGINWVR

SEQ ID NO: 63 - protein, 23 aa, Artificial Sequence
  Description of Artificial Sequence: Synthetic AX213 heavy chain CDR2 antibody region peptide
WIGRIDPGNGGTRYNEKFKGKAT

SEQ ID NO: 64 - protein, 15 aa, Artificial Sequence
  Description of Artificial Sequence: Synthetic AX213 heavy chain CDR3 antibody region peptide
CARANDGYSFDYWGQ

SEQ ID NO: 65 - protein, 108 aa, Artificial Sequence; identical to SEQ ID NO: 57
  Description of Artificial Sequence: Synthetic variable light antibody region polypeptide

SEQ ID NO: 66 - protein, 17 aa, Artificial Sequence
  Description of Artificial Sequence: Synthetic AX213 and AX132 light chain CDR1 antibody region peptide
ITCRASQYVGSYLNWYQ

SEQ ID NO: 67 - protein, 13 aa, Artificial Sequence
  Description of Artificial Sequence: Synthetic AX213 and AX132 light chain CDR2 antibody region peptide
LIYDASNRATGIP

SEQ ID NO: 68 - protein, 16 aa, Artificial Sequence
  Description of Artificial Sequence: Synthetic AX132 & AX213 light chain CDR3 antibody region peptide
YYCQVWDSSPPVVFGG

SEQ ID NO: 69 - protein, 119 aa, Artificial Sequence
  Description of Artificial Sequence: Synthetic AX1 VH antibody sequence polypeptide
EVQLLESGGGLVQPGGSLRLSCKASGFTFTSYYMHWVRQAPGKGLEWIGRINPDSGSTKYNEKFKGRATISRDNSKNTLYLQMNSLRAEDTAVYYCARGGRLSWDFDVWGQGTLVTVSS

SEQ ID NO: 70 - protein, 16 aa, Artificial Sequence
  Description of Artificial Sequence: Synthetic AX1 VH CDR1 antibody sequence peptide
KASGFTFTSYYMHWVR

SEQ ID NO: 71 - protein, 23 aa, Artificial Sequence
  Description of Artificial Sequence: Synthetic AX1 VH CDR2 antibody sequence peptide
WIGRINPDSGSTKYNEKFKGRAT

SEQ ID NO: 72 - protein, 16 aa, Artificial Sequence
  Description of Artificial Sequence: Synthetic AX1 VH CDR3 antibody sequence peptide
CARGGRLSWDFDVWGQ

SEQ ID NO: 73 - protein, 109 aa, Artificial Sequence
  Description of Artificial Sequence: Synthetic AX1 VL antibody sequence polypeptide
DIQMTQSPSSLSASVGDRVTITCRASQDISRYLAWYQQKPGKAPKLLIYAASSLQSGVPSRFSGSGSGTDFTLTISSLQPEDFATYYCAAYDYSLGGYVFGDGTKVEIK

SEQ ID NO: 74 - protein, 11 aa, Artificial Sequence
  Description of Artificial Sequence: Synthetic AX1 VL CDR1 antibody sequence peptide
RASQDISRYLA

SEQ ID NO: 75 - protein, 7 aa, Artificial Sequence
  Description of Artificial Sequence: Synthetic AX1 AX9 AX189 VL CDR2 antibody sequence peptide
AASSLQS

SEQ ID NO: 76 - protein, 11 aa, Artificial Sequence
  Description of Artificial Sequence: Synthetic AX1 VL CDR3 antibody sequence peptide
AAYDYSLGGYV

SEQ ID NO: 77 - protein, 121 aa, Artificial Sequence
  Description of Artificial Sequence: Synthetic AX9 AX189 VH antibody sequence polypeptide
EVQLLESGGGLVQPGGSLRLSCKASGYTFSSYWMHWVRQAPGKGLEWIGRIDPYNGGTKYNEKFKGKATISRDNSKNTLYLQMNSLRAEDTAVYYCARYGYYLGSYAMDYWGQGTLVTVSS

SEQ ID NO: 78 - protein, 16 aa, Artificial Sequence
  Description of Artificial Sequence: Synthetic AX9 AX189 VH CDR1 antibody sequence peptide
KASGYTFSSYWMHWVR

SEQ ID NO: 79 - protein, 23 aa, Artificial Sequence
  Description of Artificial Sequence: Synthetic AX9 AX189 VH CDR2 antibody sequence peptide
WIGRIDPYNGGTKYNEKFKGKAT

SEQ ID NO: 80 - protein, 18 aa, Artificial Sequence
  Description of Artificial Sequence: Synthetic AX9 AX189 VH CDR3 antibody sequence peptide
CARYGYYLGSYAMDYWGQ

SEQ ID NO: 81 - protein, 109 aa, Artificial Sequence
  Description of Artificial Sequence: Synthetic AX189 VL antibody sequence polypeptide
DIQMTQSPSSLSASVGDRVTITCRASQDVSRYLTWYQQKPGKAPKLLIYAASSLQSGVPSRFSGSGSGTDFTLTISSLQPEDFATYYCQAYDYSLSGYVFGGGTKVEIK

SEQ ID NO: 82 - protein, 11 aa, Artificial Sequence
  Description of Artificial Sequence: Synthetic AX189 VL CDR1 antibody sequence peptide
RASQDVSRYLT

SEQ ID NO: 83 - protein, 7 aa, Artificial Sequence
  Description of Artificial Sequence: Synthetic AX1 AX9 AX189 VL CDR2 antibody sequence peptide
AASSLQS

SEQ ID NO: 84 - protein, 11 aa, Artificial Sequence
  Description of Artificial Sequence: Synthetic AX189 VL CDR3 antibody sequence peptide
QAYDYSLSGYV

SEQ ID NO: 85 - protein, 115 aa, Homo sapiens
QVQLVQSGAEVKKPGASVKVSCKASGYTLTSYGISWVRQAPGQGLEWMGWVSFYNGNTNYAQKLQGRGTMTTDPSTSTAYMELRSLRSDDTAVYYCARGYGMDVWGQGTTVTVSS

SEQ ID NO: 86 - protein, 5 aa, Homo sapiens
SYGIS

SEQ ID NO: 87 - protein, 17 aa, Homo sapiens
WVSFYNGNTNYAQKLQG

SEQ ID NO: 88 - protein, 6 aa, Homo sapiens
GYGMDV

SEQ ID NO: 89 - protein, 109 aa, Homo sapiens
QSALTQPASVSGSPGQSITISCTGTSSDVGGYNSVSWYQQHPGKAPKLMIYEVSNRPSGVSNRFSGSKSGNTASLTISGLQAEDEADYYCNSYTSTSMVFGGGTKLTVL

SEQ ID NO: 90 - protein, 14 aa, Homo sapiens
TGTSSDVGGYNSVS

SEQ ID NO: 91 - protein, 7 aa, Homo sapiens
EVSNRPS

SEQ ID NO: 92 - protein, 9 aa, Homo sapiens
NSYTSTSMV

SEQ ID NO: 93 - protein, 123 aa, Homo sapiens
EVQLVESGGGLVKPGGSLRLSCAASGFTFSSYSMNWVRQAPGKGLEWVSSISSSSSYISYADSVKGRFTISRDNAKNSLYLQMNSLRAEDTAVYFCARDYDFWSAYYDAFDVWGQGTMVTVSS

SEQ ID NO: 94 - protein, 10 aa, Homo sapiens
GFTFSSYSMN

SEQ ID NO: 95 - protein, 17 aa, Homo sapiens
SISSSSSYISYADSVKG

SEQ ID NO: 96 - protein, 14 aa, Homo sapiens
DYDFWSAYYDAFDV

SEQ ID NO: 97 - protein, 111 aa, Homo sapiens
QSVLTQPPSVSGAPGQRVTISCTGSSSNIGAGYDVHWYQQLPGTAPKLLISGNSNRPSGVPDRFSGSKSGTSASLAITGLQAEDEADYYCQSYDSSLSGSVFGGGTKLTVL

SEQ ID NO: 98 - protein, 14 aa, Homo sapiens
TGSSSNIGAGYDVH

SEQ ID NO: 99 - protein, 7 aa, Homo sapiens
GNSNRPS

SEQ ID NO: 100 - protein, 11 aa, Homo sapiens
QSYDSSLSGSV

SEQ ID NO: 101 - protein, 114 aa, Homo sapiens
QVQLVESGGGVAQPGRSLRLSCAASGFTFSSYGMHWVRQAPGKGLEWVAVIYYDGINKHYADSVKGRFTISRDNSKNTLYLQMNSLRAEDTAVYYCARDRGLDWGQGTLVTVSS

SEQ ID NO: 102 - protein, 10 aa, Homo sapiens
GFTFSSYGMH

SEQ ID NO: 103 - protein, 17 aa, Homo sapiens
VIYYDGINKHYADSVKG

SEQ ID NO: 104 - protein, 5 aa, Homo sapiens
DRGLD

SEQ ID NO: 105 - protein, 113 aa, Homo sapiens
DIVMTQSPDSLAVSLGERATINCKSSQSVLYSSNSKNYLVWYQQKPGQPPKLLIYWASTRESGVPDRFSGSGSGTDFTLTISSLQAEDVAVYYCQQYYSTPWTFGQGTKVEIK

SEQ ID NO: 106 - protein, 17 aa, Homo sapiens
KSSQSVLYSSNSKNYLV

SEQ ID NO: 107 - protein, 7 aa, Homo sapiens
WASTRES

SEQ ID NO: 108 - protein, 9 aa, Homo sapiens
QQYYSTPWT

SEQ ID NO: 109 - protein, 118 aa, Artificial Sequence
  Description of Artificial Sequence: Synthetic anti-PCSK9 monoclonal antibody pJG04 (clones LGT-209 and LGT-210) Vh heavy chain variable region (FR1-FR4) polypeptide
QVQLVQSGAEVKKPGASVKVSCKASGYTFSTMYMSWVRQAPGQGLEWMGRIDPANEHTNYAQKFQGRVTMTRDTSISTAYMELSRLTSDDTAVYYCARSYYYYNMDYWGQGTLVTVSS

SEQ ID NO: 110 - protein, 5 aa, Artificial Sequence
  Description of Artificial Sequence: Synthetic anti-PCSK9 monoclonal antibody clones LGT-209, LGT-210 and LGT-211 heavy chain CDR1 peptide
TMYMS

SEQ ID NO: 111 - protein, 17 aa, Artificial Sequence
  Description of Artificial Sequence: Synthetic anti-PCSK9 monoclonal antibody clones LGT-209, LGT-210 and LGT-211 heavy chain CDR2 peptide
RIDPANEHTNYAQKFQG

SEQ ID NO: 112 - protein, 9 aa, Artificial Sequence
  Description of Artificial Sequence: Synthetic anti-PCSK9 monoclonal antibody pJG04(clones LGT-209 and LGT-210) Vh heavy chain complementarity determining region 3 (CDR3) peptide
SYYYYNMDY

SEQ ID NO: 113 - protein, 106 aa, Artificial Sequence
  Description of Artificial Sequence: Synthetic anti-PCSK9 monoclonal antibody pJG10(clones LGT-209 and LGT-211) Vk light chain variable region (FR1-FR4) polypeptide
QIVLTQSPATLSVSPGERATLSCRASQSVSYMHWYQQKPGQAPRLLIYGVFRRATGIPDRFSGSGSGTDFTLTIGRLEPEDFAVYYCLQWSSDPPTFGQGTKLEIK

SEQ ID NO: 114 - protein, 10 aa, Artificial Sequence
  Description of Artificial Sequence: Synthetic anti-PCSK9 monoclonal antibody clones LGT-209, LGT-210 and LGT-211 light chain CDR1 peptide
RASQSVSYMH

SEQ ID NO: 115 - protein, 7 aa, Artificial Sequence
  Description of Artificial Sequence: Synthetic anti-PCSK9 monoclonal antibody clones LGT-209, LGT-210 and LGT-211 light chain CDR1 peptide
GVFRRAT

SEQ ID NO: 116 - protein, 9 aa, Artificial Sequence
  Description of Artificial Sequence: Synthetic mouse anti-PCSK9 monoclonal antibody LFU720 and anti-PCSK9 monoclonal antibody clones LGT-209, LGT-210 and LGT-211 light chain CDR3 peptide
LQWSSDPPT

SEQ ID NO: 117 - protein, 118 aa, Homo sapiens
QVQLVQSGAEVKKPGASVKVSCKASGYTFTSYYMHWVRQAPGQGLEWMGEISPFGGRTNYNEKFKSRVTMTRDTSTSTVYMELSSLRSEDTAVYYCARERPLYASDLWGQGTTVTVSS

SEQ ID NO: 118 - protein, 7 aa, Artificial Sequence
  Description of Artificial Sequence: Synthetic peptide
GYTFTSY

SEQ ID NO: 119 - protein, 6 aa, Artificial Sequence
  Description of Artificial Sequence: Synthetic peptide
SPFGGR

SEQ ID NO: 120 - protein, 9 aa, Artificial Sequence
  Description of Artificial Sequence: Synthetic variable heavy chain CDR peptide
ERPLYASDL

SEQ ID NO: 121 - protein, 107 aa, Homo sapiens
DIQMTQSPSSLSASVGDRVTITCRASQGISSALAWYQQKPGKAPKLLIYSASYRYTGVPSRFSGSGSGTDFTFTISSLQPEDIATYYCQQRYSLWRTFGQGTKLEIK

SEQ ID NO: 122 - protein, 11 aa, Artificial Sequence
  Description of Artificial Sequence: Synthetic variable light chain CDR peptide
RASQGISSALA

SEQ ID NO: 123 - protein, 7 aa, Artificial Sequence
  Description of Artificial Sequence: Synthetic variable light chain CDR peptide
SASYRYT

SEQ ID NO: 124 - protein, 9 aa, Artificial Sequence
  Description of Artificial Sequence: Synthetic variable light chain CDR peptide
QQRYSLWRT

SEQ ID NO: 125 - protein, 118 aa, Homo sapiens
QVQLVQSGAEVKKPGASVKVSCKASGYTFTSYYMHWVRQAPGQGLEWMGEIHPSGGRTNYNEKFKSRVTMTRDTSTSTVYMELSSLRSEDTAVYYCARERPLYAMDYWGQGTTVTVSS

SEQ ID NO: 126 - protein, 10 aa, Homo sapiens
GYTFTSYYMH

SEQ ID NO: 127 - protein, 17 aa, Homo sapiens
EIHPSGGRTNYNEKFKS

SEQ ID NO: 128 - protein, 9 aa, Homo sapiens
ERPLYAMDY

SEQ ID NO: 129 - protein, 107 aa, Homo sapiens [sequence omitted]

SEQ ID NO: 130 - protein, 11 aa, Homo sapiens
KASQDVHTAVA

SEQ ID NO: 131 - protein, 7 aa, Homo sapiens
HASYRYT

SEQ ID NO: 132 - protein, 9 aa, Homo sapiens
QQRYSLWRT

SEQ ID NO: 133 - protein, 118 aa, Homo sapiens [sequence omitted]

SEQ ID NO: 134 - protein, 10 aa, Homo sapiens
GYTFTSYYMH

SEQ ID NO: 135 - protein, 17 aa, Homo sapiens
EIHPSGGRTNYNEKFKS

SEQ ID NO: 136 - protein, 9 aa, Homo sapiens
ERPLYASDL

SEQ ID NO: 137 - protein, 107 aa, Homo sapiens [sequence omitted]

SEQ ID NO: 138 - protein, 11 aa, Homo sapiens
KASQDVHTAVA

SEQ ID NO: 139 - protein, 7 aa, Homo sapiens
HASYRYT

SEQ ID NO: 140 - protein, 9 aa, Homo sapiens
QQRYSLWRT

SEQ ID NO: 141 - protein, 118 aa, Mus musculus
QVQLQQPGAELVKPGASVKLSCKASGYTFTSYWMHWVKQRPGQGLEWIGEINPSNGRTNYNEKFKSKATLTVDKSSSTAYMQLSSLTSEDSAVYYCARERPLYAMDYWGQGTSVTVSS

SEQ ID NO: 142 - protein, 7 aa, Mus musculus
GYTFTSY

SEQ ID NO: 143 - protein, 6 aa, Mus musculus
NPSNGR

SEQ ID NO: 144 - protein, 9 aa, Mus musculus
ERPLYAMDY

SEQ ID NO: 145 - protein, 108 aa, Mus musculus
DIVMTQSHKFMSTSVGDRVSITCKASQDVSTAVAWYQQKPGQSPKLLIYSASYRYTGVPDRFTGSGSGTDFTFTISSVQAEDLAVYYCQQRYSTPRTFGGGTKLEIKR

SEQ ID NO: 146 - protein, 11 aa, Mus musculus
KASQDVSTAVA

SEQ ID NO: 147 - protein, 7 aa, Artificial Sequence
  Description of Artificial Sequence: Synthetic variable light chain CDR peptide
SASYRYT

SEQ ID NO: 148 - protein, 9 aa, Mus musculus
QQRYSTPRT

SEQ ID NO: 149 - protein, 115 aa, Mus musculus
EVQLQQSGPELVKPGASVKISCKASGYTFTDYYMNWVKQSHGKSLEWIGDINPNNGGTTYNQKFKGKATLTVDKSYSTAYMELRSLTSEDSAVYYCARWLLFAYWGQGTLVTVSA

SEQ ID NO: 150 - protein, 7 aa, Mus musculus
GYTFTDY

SEQ ID NO: 151 - protein, 6 aa, Mus musculus
NPNNGG

SEQ ID NO: 152 - protein, 6 aa, Mus musculus
WLLFAY

SEQ ID NO: 153 - protein, 108 aa, Mus musculus
DIVMTQSQKFMSTSVGDRVSVTCKASQNVGTNVAWYQQKPGQSPKALIYSASYRYSGVPDRFTGSGSGTDFTLTISNVLSEDLAEYFCQQFYSYPYTFGGGTKLEIKR

SEQ ID NO: 154 - protein, 11 aa, Mus musculus
KASQNVGTNVA

SEQ ID NO: 155 - protein, 7 aa, Mus musculus
SASYRYS

SEQ ID NO: 156 - protein, 9 aa, Mus musculus
QQFYSYPYT

SEQ ID NO: 157 - protein, 123 aa, Mus musculus
EVQLQQSGPELVKPGASVKISCKASGYTFTDYYMNWVKQSHGKSLEWIGDINPNNGGTSYNQKFKGKATLTVDKSSSTAYMELRSLTSEDSAVYYCAGGGIYYRYDRNYFDYWGQGTTLTVSS

SEQ ID NO: 158 - protein, 7 aa, Mus musculus
GYTFTDY

SEQ ID NO: 159 - protein, 6 aa, Mus musculus
NPNNGG

SEQ ID NO: 160 - protein, 14 aa, Mus musculus
GGIYYRYDRNYFDY

SEQ ID NO: 161 - protein, 107 aa, Mus musculus
DIQMTQTTSSLSASLGDRVTISCSASQGISNYLNWYQQKPDGTVKLLIYYTSSLHSGVPSRFSGSGSGTDYSLTISNLEPEDIATYYCQQYSKLPFTFGSGTKLEIK

SEQ ID NO: 162 - protein, 11 aa, Mus musculus
SASQGISNYLN

SEQ ID NO: 163 - protein, 7 aa, Mus musculus
YTSSLHS

SEQ ID NO: 164 - protein, 9 aa, Artificial Sequence
  Description of Artificial Sequence: Synthetic peptide
QQYSKLPFT

SEQ ID NO: 165 - protein, 117 aa, Mus musculus
EVKLVESEGGLVQPGSSMKLSCTASGFTFSDYYMAWVRQVPEKGLEWVANINYDGSNTSYLDSLKSRFIISRDNAKNILYLQMSSLKSEDTATYYCAREKFAAMDYWGQGTSVTVSS

SEQ ID NO: 166 - protein, 7 aa, Mus musculus
GFTFSDY

SEQ ID NO: 167 - protein, 6 aa, Mus musculus
NYDGSN

SEQ ID NO: 168 - protein, 8 aa, Mus musculus
EKFAAMDY

SEQ ID NO: 169 - protein, 108 aa, Mus musculus
DIVMTQSHKFMSTSFGDRVSITCKASQDVSNALAWYQQKPGHSPKLLIFSASYRYTGVPDRFTGSGSGTDFTFTISSVQAEDLAVYYCQQHYSTPWTFGGGTKLEIKR

SEQ ID NO: 170 - protein, 11 aa, Mus musculus
KASQDVSNALA

SEQ ID NO: 171 - protein, 7 aa, Artificial Sequence
  Description of Artificial Sequence: Synthetic variable light chain CDR peptide
SASYRYT

SEQ ID NO: 172 - protein, 9 aa, Mus musculus
QQHYSTPWT

SEQ ID NO: 173 - protein, 121 aa, Artificial Sequence
  Description of Artificial Sequence: Synthetic polypeptide
EVQLVESGGGLVQPGGSLRLSCAASGFTFTRHTIHWVRQAPGKGLEWVARISPANGNTNYADSVKGRFTISADTSKNTAYLQMNSLRAEDTAVYYCARWIGSRELYIMDYWGQGTLVTVSS

SEQ ID NO: 174 - protein, 10 aa, Artificial Sequence
  Description of Artificial Sequence: Synthetic peptide
GFTFTRHTIH

SEQ ID NO: 175 - protein, 17 aa, Artificial Sequence
  Description of Artificial Sequence: Synthetic peptide
RISPANGNTNYADSVKG

SEQ ID NO: 176 - protein, 12 aa, Artificial Sequence
  Description of Artificial Sequence: Synthetic peptide
WIGSRELYIMDY

SEQ ID NO: 177 - protein, 108 aa, Artificial Sequence
  Description of Artificial Sequence: Synthetic polypeptide
DIQMTQSPSSLSASVGDRVTITCRASQDVSTAVAWYQQKPGKAPKLLIYSASFLYSGVPSRFSGSGSGTDFTLTISSLQPEDFATYYCQQSYRIQPTFGQGTKVEIKR

SEQ ID NO: 178 - protein, 11 aa, Artificial Sequence
  Description of Artificial Sequence: Synthetic peptide
RASQDVSTAVA

SEQ ID NO: 179 - protein, 7 aa, Artificial Sequence
  Description of Artificial Sequence: Synthetic peptide
SASFLYS

SEQ ID NO: 180 - protein, 9 aa, Artificial Sequence
  Description of Artificial Sequence: Synthetic peptide
QQSYRIQPT

SEQ ID NO: 181 - protein, 121 aa, Artificial Sequence
  Description of Artificial Sequence: Synthetic polypeptide
EVQLVESGGGLVQPGGSLRLSCAASGFTFSSTAIHWVRQAPGKGLEWVARISPANGNTNYADSVKGRFTISADTSKNTAYLQMNSLRAEDTAVYYCARWIGSRELYIMDYWGQGTLVTVSS

SEQ ID NO: 182 - protein, 10 aa, Artificial Sequence
  Description of Artificial Sequence: Synthetic peptide
GFTFSSTAIH

SEQ ID NO: 183 - protein, 17 aa, Artificial Sequence
  Description of Artificial Sequence: Synthetic peptide
RISPANGNTNYADSVKG

SEQ ID NO: 184 - protein, 12 aa, Artificial Sequence
  Description of Artificial Sequence: Synthetic peptide
WIGSRELYIMDY

SEQ ID NO: 185 - protein, 108 aa, Artificial Sequence
  Description of Artificial Sequence: Synthetic polypeptide
DIQMTQSPSSLSASVGDRVTITCRASQDVSTAVAWYQQKPGKAPKLLIYSASFLYSGVPSRFSGSGSGTDFTLTISSLQPEDFATYYCQQSYPALHTFGQGTKVEIKR

SEQ ID NO: 186 - protein, 11 aa, Artificial Sequence
  Description of Artificial Sequence: Synthetic peptide
RASQDVSTAVA

SEQ ID NO: 187 - protein, 7 aa, Artificial Sequence
  Description of Artificial Sequence: Synthetic peptide
SASFLYS

SEQ ID NO: 188 - protein, 9 aa, Artificial Sequence
  Description of Artificial Sequence: Synthetic peptide
QQSYPALHT

SEQ ID NO: 189 - protein, 125 aa, Artificial Sequence
  Description of Artificial Sequence: Synthetic polypeptide
EVQLVESGGGLVKPGGSLRLSCAASGFPFSKLGMVWVRQAPGKGLEWVSTISSGGGYTYYPDSVKGRFTISRDNAKNSLYLQMNSLRAEDTAVYYCAREGISFQGGTYTYVMDYWGQGTLVTVSS

SEQ ID NO: 190 - protein, 10 aa, Artificial Sequence
  Description of Artificial Sequence: Synthetic peptide
GFPFSKLGMV

SEQ ID NO: 191 - protein, 17 aa, Artificial Sequence
  Description of Artificial Sequence: Synthetic peptide
TISSGGGYTYYPDSVKG

SEQ ID NO: 192 - protein, 16 aa, Artificial Sequence
  Description of Artificial Sequence: Synthetic peptide
EGISFQGGTYTYVMDY

SEQ ID NO: 193 - protein, 112 aa, Artificial Sequence
  Description of Artificial Sequence: Synthetic polypeptide
DIVMTQSPLSLPVTPGEPASISCRSSKSLLHRNGITYSYWYLQKPGQSPQLLIYQLSNLASGVPDRFSGSGSGTDFTLKISRVEAEDVGVYYCYQNLELPLTFGQGTKVEIK

SEQ ID NO: 194 - protein, 16 aa, Artificial Sequence
  Description of Artificial Sequence: Synthetic peptide
RSSKSLLHRNGITYSY

SEQ ID NO: 195 - protein, 7 aa, Artificial Sequence
  Description of Artificial Sequence: Synthetic peptide
QLSNLAS

SEQ ID NO: 196 - protein, 9 aa, Artificial Sequence
  Description of Artificial Sequence: Synthetic peptide
YQNLELPLT

SEQ ID NO: 197 - DNA, 2076 bp, Homo sapiens
atgggcaccgtcagctccaggcggtcctggtggccgctgccactgctgctgctgctgctgctgctcctgggtcccgcgggcgcccgtgcgcaggaggacgaggacggcgactacgaggagctggtgctagccttgcgttccgaggaggacggcctggccgaagcacccgagcacggaaccacagccaccttccaccgctgcgccaaggatccgtggaggttgcctggcacctacgtggtggtgctgaaggaggagacccacctctcgcagtcagagcgcactgcccgccgcctgcaggcccaggctgcccgccggggatacctcaccaagatcctgcatgtcttccatggccttcttcctggcttcctggtgaagatgagtggcgacctgctggagctggccttgaagttgccccatgtcgactacatcgaggaggactcctctgtctttgcccagagcatcccgtggaacctggagcggattacccctccacggtaccgggcggatgaataccagccccccgacggaggcagcctggtggaggtgtatctcctagacaccagcatacagagtgaccaccgggaaatcgagggcagggtcatggtcaccgacttcgagaatgtgcccgaggaggacgggacccgcttccacagacaggccagcaagtgtgacagtcatggcacccacctggcaggggtggtcagcggccgggatgccggcgtggccaagggtgccagcatgcgcagcctgcgcgtgctcaactgccaagggaagggcacggttagcggcaccctcataggcctggagtttattcggaaaagccagctggtccagcctgtggggccactggtggtgctgctgcccctggcgggtgggtacagccgcgtcctcaacgccgcctgccagcgcctggcgagggctggggtcgtgctggtcaccgctgccggcaacttccgggacgatgcctgcctctactccccagcctcagctcccgaggtcatcacagttggggccaccaatgcccaagaccagccggtgaccctggggactttggggaccaactttggccgctgtgtggacctctttgccccaggggaggacatcattggtgcctccagcgactgcagcacctgctttgtgtcacagagtgggacatcacaggctgctgcccacgtggctggcattgcagccatgatgctgtctgccgagccggagctcaccctggccgagttgaggcagagactgatccacttctctgccaaagatgtcatcaatgaggcctggttccctgaggaccagcgggtactgacccccaacctggtggccgccctgccccccagcacccatggggcaggttggcagctgttttgcaggactgtatggtcagcacactcggggcctacacggatggccacagccgtcgcccgctgcgccccagatgaggagctgctgagctgctccagtttctccaggagtgggaagcggcggggcgagcgcatggaggcccaagggggcaagctggtctgccgggcccacaacgcttttgggggtgagggtgtctacgccattgccaggtgctgcctgctaccccaggccaactgcagcgtccacacagctccaccagctgaggccagcatggggacccgtgtccactgccaccaacagggccacgtcctcacaggctgcagctcccactgggaggtggaggaccttggcacccacaagccgcctgtgctgaggccacgaggtcagcccaaccagtgcgtgggccacagggaggccagcatccacgcttcctgctgccatgccccaggtctggaatgcaaagtcaaggagcatggaatcccggcccctcaggagcaggtgaccgtggcctgcgaggagggctggaccctgactggctgcagtgccctccctgggacctcccacgtcctgggggcctacgccgtagacaacacgtgtgtagtcaggagccgggacgtcagcactacaggcagcaccagcgaaggggccgtgacagccgttgccatctgctgccggagccggcacctggcgcaggcctcccaggagctccag

SEQ ID NO: 198 - protein, 692 aa, Homo sapiens
MGTVSSRRSWWPLPLLLLLLLLLGPAGARAQEDEDGDYEELVLALRSEEDGLAEAPEHGTTATFHRCAKDPWRLPGTYVVVLKEETHLSQSERTARRLQAQAARRGYLTKILHVFHGLLPGFLVKMSGDLLELALKLPHVDYIEEDSSVFAQSIPWNLERITPPRYRADEYQPPDGGSLVEVYLLDTSIQSDHREIEGRVMVTDFENVPEEDGTRFHRQASKCDSHGTHLAGVVSGRDAGVAKGASMRSLRVLNCQGKGTVSGTLIGLEFIRKSQLVQPVGPLVVLLPLAGGYSRVLNAACQRLARAGVVLVTAAGNFRDDACLYSPASAPEVITVGATNAQDQPVTLGTLGTNFGRCVDLFAPGEDIIGASSDCSTCFVSQSGTSQAAAHVAGIAAMMLSAEPELTLAELRQRLIHFSAKDVINEAWFPEDQRVLTPNLVAALPPSTHGAGWQLFCRTVWSAHSGPTRMATAVARCAPDEELLSCSSFSRSGKRRGERMEAQGGKLVCRAHNAFGGEGVYAIARCCLLPQANCSVHTAPPAEASMGTRVHCHQQGHVLTGCSSHWEVEDLGTHKPPVLRPRGQPNQCVGHREASIHASCCHAPGLECKVKEHGIPAPQEQVTVACEEGWTLTGCSALPGTSHVLGAYAVDNTCVVRSRDVSTTGSTSEGAVTAVAICCRSRHLAQASQELQ